European Patent Application EP 4 442 366 A2, published October 9, 2024. Title: METHODS FOR FAST NUCLEIC ACID AMPLIFICATION. Applicant: University of Utah Research Foundation. The sequence listing filed with the application follows.

SEQUENCE LISTING (27 sequences)

SEQ ID NO: 1 - DNA, 24 bp, Homo sapiens
  source 1..24: mol_type = other DNA
cccattcaacgtctacatcgagtc

SEQ ID NO: 2 - DNA, 19 bp, Homo sapiens
  source 1..19: mol_type = other DNA
tccttctcttgccaggcat

SEQ ID NO: 3 - DNA, 45 bp, Homo sapiens
  variation 23: note = mutation - G or A residue
  source 1..45: mol_type = other DNA
cccattcaacgtctacatcgagtccgatgcctggcaagagaagga

SEQ ID NO: 4 - DNA, 20 bp, Homo sapiens
  source 1..20: mol_type = other DNA
ctacagtgggagtcacctgc

SEQ ID NO: 5 - DNA, 25 bp, Homo sapiens
  source 1..25: mol_type = other DNA
ggtactgagctgtgaaagtcaggtt

SEQ ID NO: 6 - DNA, 58 bp, Homo sapiens
  variation 28: note = mutation - A or G residue
  source 1..58: mol_type = other DNA
ctacagtgggagtcacctgcttttgccaaagggaacctgactttcacagctcagtacc

SEQ ID NO: 7 - DNA, 20 bp, Homo sapiens
  source 1..20: mol_type = other DNA
gggagtcacctgcttttgcc

SEQ ID NO: 8 - DNA, 25 bp, Homo sapiens
  source 1..25: mol_type = other DNA
tactgagctgtgaaagtcaggttcc

SEQ ID NO: 9 - DNA, 49 bp, Homo sapiens
  source 1..49: mol_type = other DNA
gggagtcacctgcttttgccaaagggaacctgactttcacagctcagta

SEQ ID NO: 10 - DNA, 34 bp, Homo sapiens
  source 1..34: mol_type = other DNA
ctctgtgctttctgtatcctcagagtggcattct

SEQ ID NO: 11 - DNA, 28 bp, Homo sapiens
  source 1..28: mol_type = other DNA
cgtctgctggagtgtgcccaatgctata

SEQ ID NO: 12 - DNA, 60 bp, Homo sapiens
  misc_feature 1..41: note = 5' standard synthetic region
  source 1..60: mol_type = other DNA
acacacacacacacacacacacacacacacacacacaaaaattcagtggcattaaatacg

SEQ ID NO: 13 - DNA, 67 bp, Homo sapiens
  misc_feature 1..50: note = 5' standard synthetic region
  source 1..67: mol_type = other DNA
gagagagagagagagagagagagagagagagagagagagagagagaaaaaccagagctaaagggaag

SEQ ID NO: 14 - DNA, 66 bp, Homo sapiens
  misc_feature 1..41: note = 5' standard synthetic region
  source 1..66: mol_type = other DNA
acacacacacacacacacacacacacacacacacacaaaaagctggtgtctgctatagaactgatt

SEQ ID NO: 15 - DNA, 72 bp, Homo sapiens
  misc_feature 1..50: note = 5' standard synthetic region
  source 1..72: mol_type = other DNA
gagagagagagagagagagagagagagagagagagagagagagagaaaaagttgccagagctaaagggaagg

SEQ ID NO: 16 - DNA, 41 bp, synthetic construct
  misc_feature 1..41: note = Synthetic common primer
  source 1..41: mol_type = other DNA
acacacacacacacacacacacacacacacacacacaaaaa

SEQ ID NO: 17 - DNA, 50 bp, synthetic construct
  misc_feature 1..50: note = Synthetic common primer
  source 1..50: mol_type = other DNA
gagagagagagagagagagagagagagagagagagagagagagagaaaaa

SEQ ID NO: 18 - DNA, 24 bp, synthetic construct
  misc_feature 1..24: note = Synthetic common primer
  source 1..24: mol_type = other DNA
actcgcacgaactcaccgcactcc

SEQ ID NO: 19 - DNA, 24 bp, synthetic construct
  misc_feature 1..24: note = Synthetic common primer
  source 1..24: mol_type = other DNA
actcgcacgaactcaccgcactcc

SEQ ID NO: 20 - DNA, 100 bp, synthetic construct
  misc_feature 1..100: note = Synthetic template
  source 1..100: mol_type = other DNA
actcgcacgaactcaccgcactccggatggattgtgaagaggcccaagatactggtcatattatcctttgatctagctctcactcgcactctcacgcaca

SEQ ID NO: 21 - DNA, 200 bp, synthetic construct
  misc_feature 1..200: note = Synthetic template
  source 1..200: mol_type = other DNA
actcgcacgaactcaccgcactcctcaatgctgacaaatcgaaagaataggaatagcgtaattactagaggactccaatatagtatattaccctggtgaccgcctgtactgtaggaacactaccgcggttatattgacagcttagcaatctaccctgttgggatctgtttaagtggctctcactcgcactctcacgcaca

SEQ ID NO: 22 - DNA, 300 bp, synthetic construct
  misc_feature 1..300: note = Synthetic template
  source 1..300: mol_type = other DNA
actcgcacgaactcaccgcactccccttcgaatataaagtacgacattactagcaatgacagttccaggatttaagaaagtagtgttccacatcaatgcatatccagtgaaagcataacgtcaaaaaaagcctggcaccgttcgcgatctggacttacttagatttgttgtagtcaagccggctatcagcgatttatcccggaaacacatactagtgagttatttgtatgttacctagaatagctgtcacgaatcactaatacattcacccaccagctctcactcgcactctcacgcaca

SEQ ID NO: 23 - DNA, 400 bp, synthetic construct
  misc_feature 1..400: note = Synthetic template
  source 1..400: mol_type = other DNA
actcgcacgaactcaccgcactcctgaatacaagacgacagtcctgattatattttcatttaattacgccaatttaattatgatgaatattaacggaattaaatatgtattgataagtactaagtaatggtttacccacggcgatctatatgcaagggaaacattaacaaatttaaacatctgatgtggacaaaacttgtaatgtggtatagttaaaaatataggtttcagggacacgtaagtatctatcttgaatgtttaagtaggtcctgtctaccattctgaaatttagaaaatcgcgttcatcgggctgtcggctacacctcagaaaaccatttcgtgttgcacaggaggaactttcgagggttcgtatgagctctcactcgcactctcacgcaca

SEQ ID NO: 24 - DNA, 500 bp, synthetic construct
  misc_feature 1..500: note = Synthetic template
  source 1..500: mol_type = other DNA
actcgcacgaactcaccgcactccaccgcttgacgacgtagggtatttggtatctgaatctactcatttacctacatactgaagattttgcgatcgtctaatatattggactaatgcccgatttctgatcaattactctaggcgatacttcatcgctggccttatttggattttgctcaagtgctaaactctctgcgcgtcaatactagtctgacatcagtcaagacctgctatctgaaaactactagagagatatacctaacaactttagtggataaatcaggtctggagattgtcatataatgccactagggtcagaaggctgtgtcaaagttagtggttagtaggtctccgctctgcggtactattcttatattctcttactatgcatcaaacaaaatagaatgcatagacaaaccgcctgccaagtttacaagataacttgcgtataggtttataagggttcttctgtatcgctctcactcgcactctcacgcaca

SEQ ID NO: 25 - DNA, 31 bp, Homo sapiens
  source 1..31: mol_type = other DNA
gcttggaagattgctaaaatgatagtcagtg

SEQ ID NO: 26 - DNA, 26 bp, Homo sapiens
  source 1..26: mol_type = other DNA
ttgatcatactgagcctgctgcataa

SEQ ID NO: 27 - DNA, 60 bp, Homo sapiens
  variation 34: note = mutation - A or G residue
  source 1..60: mol_type = other DNA
gcttggaagattgctaaaatgatagtcagtgacattatgcagcaggctcagtatgatcaa